European Patent Application EP 4 488 281 A1, published January 8, 2025. Title: 5' position modified nucleoside and nucleotide using the same. Applicant: Osaka University. Application WO. The sequence listing filed with the application follows.

SEQUENCE LISTING (28 sequences)

SEQ ID NO: 1 - DNA, 12 bp, synthetic construct
  misc_feature 1..12: note = SSO(unmodified)
  source 1..12: mol_type = other DNA
gcgttttttgct

SEQ ID NO: 2 - DNA, 12 bp, synthetic construct
  misc_feature 1..12: note = SSO(5'-cp)
  modified_base 6: mod_base = OTHER; note = t = 5'-cyclopropanethymidine
  source 1..12: mol_type = other DNA
gcgttttttgct

SEQ ID NO: 3 - DNA, 12 bp, synthetic construct
  misc_feature 1..12: note = SSO(5'-cp2)
  modified_base 6: mod_base = OTHER; note = t = 5'-cyclopententhymidine
  source 1..12: mol_type = other DNA
gcgttttttgct

SEQ ID NO: 4 - DNA, 12 bp, synthetic construct
  misc_feature 1..12: note = SSO(5'-cp3)
  modified_base 6: mod_base = OTHER; note = t = 5'-cyclopentanthymidine
  source 1..12: mol_type = other DNA
gcgttttttgct

SEQ ID NO: 5 - DNA, 12 bp, synthetic construct
  misc_feature 1..12: note = SSO(3 x 5'-cp3_1)
  modified_base 5: mod_base = OTHER; note = t = 5'-cyclopentanthymidine
  modified_base 7: mod_base = OTHER; note = t = 5'-cyclopentanthymidine
  modified_base 9: mod_base = OTHER; note = t = 5'-cyclopentanthymidine
  source 1..12: mol_type = other DNA
gcgttttttgct

SEQ ID NO: 6 - DNA, 12 bp, synthetic construct
  misc_feature 1..12: note = SSO(3 x 5'-cp3_2)
  modified_base 5..7: mod_base = OTHER; note = t = 5'-cyclopentanthymidine
  source 1..12: mol_type = other DNA
gcgttttttgct

SEQ ID NO: 7 - DNA, 10 bp, synthetic construct
  misc_feature 1..10: note = SSO_all T(unmodified)
  source 1..10: mol_type = other DNA
tttttttttt

SEQ ID NO: 8 - DNA, 10 bp, synthetic construct
  misc_feature 1..10: note = SSO_all T(PS)
  modified_base 10: mod_base = OTHER; note = phosphorotioated
  source 1..10: mol_type = other DNA
tttttttttt

SEQ ID NO: 9 - DNA, 10 bp, synthetic construct
  misc_feature 1..10: note = SSO_all T(5'-cp)
  modified_base 10: mod_base = OTHER; note = t = 5'-cyclopropanethymidine
  source 1..10: mol_type = other DNA
tttttttttt

SEQ ID NO: 10 - DNA, 10 bp, synthetic construct
  misc_feature 1..10: note = SSO_all T(cp2)
  modified_base 10: mod_base = OTHER; note = t = 5'-cyclopententhymidine
  source 1..10: mol_type = other DNA
tttttttttt

SEQ ID NO: 11 - DNA, 10 bp, synthetic construct
  misc_feature 1..10: note = SSO_all T(5'-cp3)
  modified_base 10: mod_base = OTHER; note = t = 5'-cyclopentanthymidine
  source 1..10: mol_type = other DNA
tttttttttt

SEQ ID NO: 12 - DNA, 20 bp, synthetic construct
  misc_feature 1..20: note = PCR Primer(NR3C1 forward)
  source 1..20: mol_type = other DNA
actgtccagcatgccgctat

SEQ ID NO: 13 - DNA, 20 bp, synthetic construct
  misc_feature 1..20: note = PCR Primer(NR3C1 reverse)
  source 1..20: mol_type = other DNA
gcagtggcttgctgaattcc

SEQ ID NO: 14 - DNA, 20 bp, synthetic construct
  misc_feature 1..20: note = PCR Primer(GAPDH forward)
  source 1..20: mol_type = other DNA
gtgtgaacggatttggccgt

SEQ ID NO: 15 - DNA, 20 bp, synthetic construct
  misc_feature 1..20: note = PCR Primer(GAPDH reverse)
  source 1..20: mol_type = other DNA
gacaagcttcccattctcgg

SEQ ID NO: 16 - DNA, 14 bp, synthetic construct
  misc_feature 1..14: note = Posi12
  modified_base 1: mod_base = OTHER; note = g = LNA-G
  modified_base 2: mod_base = OTHER; note = t = LNA-T
  modified_base 2..14: mod_base = OTHER; note = phosphorotioated
  modified_base 3: mod_base = OTHER; note = c = LNA-5-methylcytidine
  modified_base 12: mod_base = OTHER; note = t = LNA-T
  modified_base 13: mod_base = OTHER; note = g = LNA-G
  modified_base 14: mod_base = OTHER; note = g = LNA-G
  source 1..14: mol_type = other DNA
gtctctttacctgg

SEQ ID NO: 17 - DNA, 14 bp, synthetic construct
  misc_feature 1..14: note = Posi12-4cp3
  modified_base 1: mod_base = OTHER; note = g = LNA-G
  modified_base 2: mod_base = OTHER; note = t = LNA-T
  modified_base 2..14: mod_base = OTHER; note = phosphorotioated
  modified_base 3: mod_base = OTHER; note = c = LNA-5-methylcytidine
  modified_base 4: mod_base = OTHER; note = t = 5'-cp3-T
  modified_base 12: mod_base = OTHER; note = t = LNA-T
  modified_base 13: mod_base = OTHER; note = g = LNA-G
  modified_base 14: mod_base = OTHER; note = g = LNA-G
  source 1..14: mol_type = other DNA
gtctctttacctgg

SEQ ID NO: 18 - DNA, 14 bp, synthetic construct
  misc_feature 1..14: note = Posi12-7cp3
  modified_base 1: mod_base = OTHER; note = g = LNA-G
  modified_base 2: mod_base = OTHER; note = t = LNA-T
  modified_base 2..14: mod_base = OTHER; note = phosphorotioated
  modified_base 3: mod_base = OTHER; note = c = LNA-5-methylcytidine
  modified_base 7: mod_base = OTHER; note = t = 5'-cp3-T
  modified_base 12: mod_base = OTHER; note = t = LNA-T
  modified_base 13: mod_base = OTHER; note = g = LNA-G
  modified_base 14: mod_base = OTHER; note = g = LNA-G
  source 1..14: mol_type = other DNA
gtctctttacctgg

SEQ ID NO: 19 - RNA, 12 nt, synthetic construct
  misc_feature 1..12: note = target ssRNA sequence
  source 1..12: mol_type = other RNA
agcaaaaaacgc

SEQ ID NO: 20 - DNA, 12 bp, synthetic construct
  misc_feature 1..12: note = SSO(unmodified)
  source 1..12: mol_type = other DNA
gcgttctttgct

SEQ ID NO: 21 - DNA, 12 bp, synthetic construct
  misc_feature 1..12: note = SSO(5'-cp-5-methylcytosine)
  modified_base 6: mod_base = OTHER; note = c = 5'-cyclopropane-5-methylcytosine
  source 1..12: mol_type = other DNA
gcgttctttgct

SEQ ID NO: 22 - DNA, 12 bp, synthetic construct
  misc_feature 1..12: note = SSO(unmodified)
  source 1..12: mol_type = other DNA
gcgttatttgct

SEQ ID NO: 23 - DNA, 12 bp, synthetic construct
  misc_feature 1..12: note = SSO(5'-cyclopropaneadenine)
  modified_base 6: mod_base = OTHER; note = a = 5'-cyclopropaneadenine
  source 1..12: mol_type = other DNA
gcgttatttgct

SEQ ID NO: 24 - DNA, 12 bp, synthetic construct
  misc_feature 1..12: note = SSO(unmodified)
  source 1..12: mol_type = other DNA
gcgttgtttgct

SEQ ID NO: 25 - DNA, 12 bp, synthetic construct
  misc_feature 1..12: note = SSO(5'-cyclopropaneguanine)
  modified_base 6: mod_base = OTHER; note = g = 5'-cyclopropaneguanine
  source 1..12: mol_type = other DNA
gcgttgtttgct

SEQ ID NO: 26 - RNA, 12 nt, synthetic construct
  misc_feature 1..12: note = target ssRNA sequence
  source 1..12: mol_type = other RNA
agcaaagaacgc

SEQ ID NO: 27 - RNA, 12 nt, synthetic construct
  misc_feature 1..12: note = target ssRNA sequence
  source 1..12: mol_type = other RNA
agcaaataacgc

SEQ ID NO: 28 - RNA, 12 nt, synthetic construct
  misc_feature 1..12: note = target ssRNA sequence
  source 1..12: mol_type = other RNA
agcaaacaacgc